European Patent Specification EP 3 831 836 B1, published September 6, 2023. Title: Compound or salt thereof and anti-adenovirus agent. Applicant: FUJIFILM Corporation. The sequence listing filed with the application follows.

SEQUENCE LISTING (2 sequences)

SEQ ID NO: 1 - DNA, 17 bp, Artificial Sequence
  Description of Artificial Sequence: oligonucleotide
gtaaaacgacggccagt

SEQ ID NO: 2 - DNA, 70 bp, Artificial Sequence
  Description of Artificial Sequence: oligonucleotide
ccggggatcctctagagtcgacctgcaggcatgcaagcttggcactggccgtcgttttacaacgtcgtga